European Patent Application EP 4 446 417 A1, published October 16, 2024. Title: Mutant of Corynebacterium glutamicum with enhanced L-lysine productivity and method for preparing L-lysine using the same. Applicant: DAESANG CORPORATION. The sequence listing filed with the application follows.

SEQUENCE LISTING (16 sequences)

SEQ ID NO: 1 - protein, 334 aa, Corynebacterium sp.
MTIRVGINGFGRIGRNFFRAVLERSDDLEVVAVNDLTDNKTLSTLLKFDSIMGRLGQEVEYDDDSITVGGKRIAVYAERDPKNLDWAAHNVDIVIESTGFFTDANAAKAHIEAGAKKVIISAPASNEDATFVYGVNHESYDPENHNVISGASCTTNCLAPMAKVLNDKFGIENGLMTTVHAYTGDQRLHDAPHRDLRRARAAAVNIVPTSTGAAKAVALVLPELKGKLDGYALRVPVITGSATDLTFNTKSEVTVESINAAIKEAAVGEFGETLAYSEEPLVSTDIVHDSHGSIFDAGLTKVSGNTVKVVSWYDNEWGYTCQLLRLTELVASKL

SEQ ID NO: 2 - DNA, 1005 bp, Corynebacterium sp.
  source 1..1005: mol_type = genomic DNA
atgaccattcgtgttggtattaacggatttggccgtatcggacgtaacttcttccgcgcagttctggagcgcagcgacgatctcgaggtagttgcagtcaacgacctcaccgacaacaagaccctttccacccttctcaagttcgactccatcatgggccgccttggccaggaagttgaatacgacgatgactccatcaccgttggtggcaagcgcatcgctgtttacgcagagcgcgatccaaagaacctggactgggctgcacacaacgttgacatcgtgatcgagtccaccggcttcttcaccgatgcaaacgcggctaaggctcacatcgaagcaggtgccaagaaggtcatcatctccgcaccagcaagcaacgaagacgcaaccttcgtttacggtgtgaaccacgagtcctacgatcctgagaaccacaacgtgatctccggcgcatcttgcaccaccaactgcctcgcaccaatggcaaaggtcctaaacgacaagttcggcatcgagaacggcctcatgaccaccgttcacgcatacactggcgaccagcgcctgcacgatgcacctcaccgcgacctgcgtcgtgcacgtgcagcagcagtcaacatcgttcctacctccaccggtgcagctaaggctgttgctctggttctcccagagctcaagggcaagcttgacggctacgcacttcgcgttccagttatcaccggttccgcaaccgacctgaccttcaacaccaagtctgaggtcaccgttgagtccatcaacgctgcaatcaaggaagctgcagtcggcgagttcggcgagaccctggcttactccgaagagccactggtttccaccgacatcgtccacgattcccacggctccatcttcgacgctggcctgaccaaggtctccggcaacaccgtcaaggttgtttcctggtacgacaacgagtggggctacacctgccagctcctgcgtctgaccgagctcgtagcttccaagctctaa

SEQ ID NO: 3 - protein, 334 aa, synthetic construct
MTIRVGINGFGRIGRNFFRAVLERSDDLEVVAVNDSKDNKTLSTLLKFDSIMGRLGQEVEYDDDSITVGGKRIAVYAERDPKNLDWAAHNVDIVIESTGFFTDANAAKAHIEAGAKKVIISAPASNEDATFVYGVNHESYDPENHNVISGASCTTNCLAPMAKVLNDKFGIENGLMTTVHAYTGDQRLHDAPHRDLRRARAAAVNIVPTSTGAAKAVALVLPELKGKLDGYALRVPVITGSATDLTFNTKSEVTVESINAAIKEAAVGEFGETLAYSEEPLVSTDIVHDSHGSIFDAGLTKVSGNTVKVVSWYDNEWGYTCQLLRLTELVASKL

SEQ ID NO: 4 - DNA, 1005 bp, synthetic construct
  source 1..1005: mol_type = other DNA
atgaccattcgtgttggtattaacggatttggccgtatcggacgtaacttcttccgcgcagttctggagcgcagcgacgatctcgaggtagttgcagtcaacgactccaaggacaacaagaccctttccacccttctcaagttcgactccatcatgggccgccttggccaggaagttgaatacgacgatgactccatcaccgttggtggcaagcgcatcgctgtttacgcagagcgcgatccaaagaacctggactgggctgcacacaacgttgacatcgtgatcgagtccaccggcttcttcaccgatgcaaacgcggctaaggctcacatcgaagcaggtgccaagaaggtcatcatctccgcaccagcaagcaacgaagacgcaaccttcgtttacggtgtgaaccacgagtcctacgatcctgagaaccacaacgtgatctccggcgcatcttgcaccaccaactgcctcgcaccaatggcaaaggtcctaaacgacaagttcggcatcgagaacggcctcatgaccaccgttcacgcatacactggcgaccagcgcctgcacgatgcacctcaccgcgacctgcgtcgtgcacgtgcagcagcagtcaacatcgttcctacctccaccggtgcagctaaggctgttgctctggttctcccagagctcaagggcaagcttgacggctacgcacttcgcgttccagttatcaccggttccgcaaccgacctgaccttcaacaccaagtctgaggtcaccgttgagtccatcaacgctgcaatcaaggaagctgcagtcggcgagttcggcgagaccctggcttactccgaagagccactggtttccaccgacatcgtccacgattcccacggctccatcttcgacgctggcctgaccaaggtctccggcaacaccgtcaaggttgtttcctggtacgacaacgagtggggctacacctgccagctcctgcgtctgaccgagctcgtagcttccaagctctaa

SEQ ID NO: 5 - protein, 334 aa, synthetic construct
MTIRVGINGFGRIGRNFFRAVLERSDDLEVVAVNDSKDNKTLSTLLKFDSIMGRLGQEVEYDDDSITVGGKRIAVYAERDPKNLDWAAHNVDIVIESTGVFTDANAAKAHIEAGAKKVIISAPASNEDATFVYGVNHESYDPENHNVISGASCTTNCLAPMAKVLNDKFGIENGLMTTVHAYTGDQRLHDAPHRDLRRARAAAVNIVPTSTGAAKAVALVLPELKGKLDGYALRVPVITGSATDLTFNTKSEVTVESINAAIKEAAVGEFGETLAYSEEPLVSTDIVHDSHGSIFDAGLTKVSGNTVKVVSWYDNEWGYTCQLLRLTELVASKL

SEQ ID NO: 6 - DNA, 1005 bp, synthetic construct
  source 1..1005: mol_type = other DNA
atgaccattcgtgttggtattaacggatttggccgtatcggacgtaacttcttccgcgcagttctggagcgcagcgacgatctcgaggtagttgcagtcaacgactccaaggacaacaagaccctttccacccttctcaagttcgactccatcatgggccgccttggccaggaagttgaatacgacgatgactccatcaccgttggtggcaagcgcatcgctgtttacgcagagcgcgatccaaagaacctggactgggctgcacacaacgttgacatcgtgatcgagtccaccggcgtcttcaccgatgcaaacgcggctaaggctcacatcgaagcaggtgccaagaaggtcatcatctccgcaccagcaagcaacgaagacgcaaccttcgtttacggtgtgaaccacgagtcctacgatcctgagaaccacaacgtgatctccggcgcatcttgcaccaccaactgcctcgcaccaatggcaaaggtcctaaacgacaagttcggcatcgagaacggcctcatgaccaccgttcacgcatacactggcgaccagcgcctgcacgatgcacctcaccgcgacctgcgtcgtgcacgtgcagcagcagtcaacatcgttcctacctccaccggtgcagctaaggctgttgctctggttctcccagagctcaagggcaagcttgacggctacgcacttcgcgttccagttatcaccggttccgcaaccgacctgaccttcaacaccaagtctgaggtcaccgttgagtccatcaacgctgcaatcaaggaagctgcagtcggcgagttcggcgagaccctggcttactccgaagagccactggtttccaccgacatcgtccacgattcccacggctccatcttcgacgctggcctgaccaaggtctccggcaacaccgtcaaggttgtttcctggtacgacaacgagtggggctacacctgccagctcctgcgtctgaccgagctcgtagcttccaagctctaa

SEQ ID NO: 7 - DNA, 19 bp, synthetic construct
  source 1..19: mol_type = other DNA
agtgcgaacgatttcaggt

SEQ ID NO: 8 - DNA, 34 bp, synthetic construct
  source 1..34: mol_type = other DNA
gaccatgattacgccagtgcgaacgatttcaggt

SEQ ID NO: 9 - DNA, 20 bp, synthetic construct
  source 1..20: mol_type = other DNA
ggagtcgttgactgcaacta

SEQ ID NO: 10 - DNA, 20 bp, synthetic construct
  source 1..20: mol_type = other DNA
actgcaactacctcgagatc

SEQ ID NO: 11 - DNA, 20 bp, synthetic construct
  source 1..20: mol_type = other DNA
aaggacaacaagaccctttc

SEQ ID NO: 12 - DNA, 30 bp, synthetic construct
  source 1..30: mol_type = other DNA
caacgactccaaggacaacaagaccctttc

SEQ ID NO: 13 - DNA, 20 bp, synthetic construct
  source 1..20: mol_type = other DNA
aaccagagcaacagccttag

SEQ ID NO: 14 - DNA, 20 bp, synthetic construct
  source 1..20: mol_type = other DNA
acagccttagctgcaccggt

SEQ ID NO: 15 - DNA, 19 bp, synthetic construct
  source 1..19: mol_type = other DNA
ttcaccgatgcaaacgcgg

SEQ ID NO: 16 - DNA, 29 bp, synthetic construct
  source 1..29: mol_type = other DNA
caccggcgtcttcaccgatgcaaacgcgg